European Patent Specification EP 3 363 284 B1, published April 8, 2026. Title: METHODS AND COMPOSITIONS FOR WATERMELON SEX EXPRESSION. Applicant: Seminis Vegetable Seeds, Inc. The sequence listing filed with the application follows.

SEQUENCE LISTING (13 sequences)

SEQ ID NO: 1 - DNA, 121 bp, Citrullus lanatus
  misc_feature (12)..(12): n is a, c, g, or t
  misc_feature (17)..(17): n is a, c, g, or t
  misc_feature (105)..(105): n is a, c, g, or t
tgttgttaaaangaaancagataggggtaggggtagccgacagattgcaacagtttgctgyccagtgttattaaagccacacctaggcatggtttccaaaaaaangtgttgaaaagtgacg

SEQ ID NO: 2 - DNA, 121 bp, Citrullus lanatus
tatgtagtagatacattagtccagggatgtaatgtacctaggcgagactttactaattccrgtgcggccaacagatgacaacggggaaccaggagatggtgaatcactattaggtgaagtt

SEQ ID NO: 3 - DNA, 121 bp, Citrullus lanatus
atgcacatccaaccctgtctgaggtgcttgatgaactatttaaatcagccaaggtcagttyaacatttttgtagatcatgcttgacctacaagactagttcctatgtcaatggaatccaac

SEQ ID NO: 4 - DNA, 120 bp, Citrullus lanatus
ggattatttgggtcctttaacttcaagtgggtggagtaggctattatagctttgagactcygattataattgttagtgttttcaactattataacctacaactaactacaatattactgt

SEQ ID NO: 5 - DNA, 121 bp, Citrullus lanatus
tcgagcaaatgaagagtatggctggaaaacataaagatgattctggtgaaggttcggagcstacttcgcagatcaaactgacggtggacgagttcgaatcattgagcagaaaggtcagaga

SEQ ID NO: 6 - DNA, 121 bp, Citrullus lanatus
  misc_feature (79)..(79): n is a, c, g, or t
aataatattttaaagggacaacgcatctgatggctagcttttgcgtttctccttattaatwaaggagtcttgataaaancaatctttcaatctttaactcttcctgagaattaggatcgcg

SEQ ID NO: 7 - DNA, 121 bp, Citrullus lanatus
ctatagtgcagctgcacgtccgcaaccggctctatattttctacgagcagattctagcttygaacctcatcgaaaatgcgtccaatcttgatgaaaggccatgaacggccattaactttcc

SEQ ID NO: 8 - DNA, 121 bp, Citrullus lanatus
agattaccgattaataactaggcaacattggcttgcccattgcttgttatggttccaggcmaacctggccgcacaccatatttagttattttatcgatttctttctttgacattacttctt

SEQ ID NO: 9 - DNA, 121 bp, Citrullus lanatus
cagactgttggcaaatattgtttggcacctccatttcgagatagaaagctgtttagcaagstgttattttcatcacactacagaatatttggttgaaaaggaactagagaatgtctcatga

SEQ ID NO: 10 - DNA, 121 bp, Citrullus lanatus
  misc_feature (98)..(98): n is a, c, g, or t
  misc_feature (112)..(113): n is a, c, g, or t
tcctgcgcatcctatcaggacctccactcatggagatggcggagagggttgggagagcggmaagcacagggcagttgagtttcaggcatttgaagaangaaagtgatggtgnnaatgaagg

SEQ ID NO: 11 - DNA, 120 bp, Citrullus lanatus
  misc_feature (94)..(95): n is a, c, g, or t
  misc_feature (99)..(99): n is a, c, g, or t
tgagataagatgggatgatcacgggatgactcagcttttgttcaaagcttccacctatttkctattctattttccttaatttgtttaaaaaatnnctcntctatattttcgaaaattaca

SEQ ID NO: 12 - DNA, 121 bp, Citrullus lanatus
  misc_feature (34)..(34): n is a, c, g, or t
  misc_feature (38)..(38): n is a, c, g, or t
aataaggtgaaaggactagaccagggtttaagcnaaantcctggagctactcaagcatccmaaccccatcatggaaaccttggcaaaggtggctgaagagtaccccgagggtagccggcgt

SEQ ID NO: 13 - DNA, 121 bp, Citrullus lanatus
ctgatcattcccaaaacttcggtttgtctcttgagaaccctgagcttctcccggttggcarggatgaatttgtttgccaaacttctcaagttcttgcacttcattttgggcatgatagtct